European Patent Application EP 4 174 088 A1, published May 3, 2023. Title: FUSION PROTEIN COMPRISING ANTI-LAG-3 ANTIBODY AND IL-2 AND USE THEREOF. Applicant: GI Innovation, Inc. The sequence listing filed with the application follows.

SEQUENCE LISTING (29 sequences)

SEQ ID NO: 1 - protein, 8 aa, Artificial Sequence
  VH-CDR1 of anti-hLAG3 (1E09)
GFSFSDHY

SEQ ID NO: 2 - protein, 8 aa, Artificial Sequence
  VH-CDR2 of anti-hLAG3 (1E09)
IDTSATYI

SEQ ID NO: 3 - protein, 10 aa, Artificial Sequence
  VH-CDR3 of anti-hLAG3 (1E09)
ARDNWGSLDY

SEQ ID NO: 4 - protein, 117 aa, Artificial Sequence
  Variable heavy chain of anti-hLAG3 (1E09)
QVQLVQSGGDLVKPGGSLRLSCAASGFSFSDHYMNWIRQAPGKGLEWVAYIDTSATYIYYADSVKGRFTISRDNAKNSLYLQMNSLRAEDTAVYYCARDNWGSLDYWGQGALVTVSS

SEQ ID NO: 5 - protein, 6 aa, Artificial Sequence
  VL-CDR1 of anti-hLAG3 (1E09)
QEISIY

SEQ ID NO: 6 - protein, 3 aa, Artificial Sequence
  VL-CDR2 of anti-hLAG3 (1E09)
DAS

SEQ ID NO: 7 - protein, 9 aa, Artificial Sequence
  VL-CDR3 of anti-hLAG3 (1E09)
QQTYITPYT

SEQ ID NO: 8 - protein, 107 aa, Artificial Sequence
  Variable light chain of anti-hLAG3 (1E09)
DIQMTQSPSSLSPSVGDRVTITCQASQEISIYLNWYQQKPGKAPKLLIYDASNLETGVPSRFSGSGSGTDFTLTISSLQPEDFATYYCQQTYITPYTFGQGTKLDIK

SEQ ID NO: 9 - DNA, 351 bp, Artificial Sequence
  Variable heavy chain gene of anti-hLAG3 (1E09)
caggttcagttggttcagtctggcggcgacctggttaagcctggcggatctctgagactgtcttgtgccgcctccggcttctccttctccgaccactacatgaactggatcagacaggcccctggcaaaggcctggaatgggtcgcctacatcgatacctccgccacctacatctactacgccgactccgtgaagggcagattcaccatctccagagacaacgccaagaactccctgtacctccagatgaacagcctgagagccgaggacaccgccgtgtactactgcgccagagataactggggctccctggattattggggccagggcgctctggtcacagtgtcctct

SEQ ID NO: 10 - DNA, 321 bp, Artificial Sequence
  Variable light chain gene of anti-hLAG3 (1E09)
gacattcagatgacccagtctccatcctctctgagcccatccgtgggcgacagagtgaccattacctgccaggccagccaagagatctccatctacctgaactggtatcagcagaagcccggcaaggcccctaagctgctgatctacgacgcctccaatctggaaacaggcgtgccctccagattctccggctctggctctggcacagactttaccctgaccatctccagcctccagcctgaggatttcgccacctactactgccagcagacctacatcaccccttacacctttggccagggcaccaagctggacatcaag

SEQ ID NO: 11 - protein, 367 aa, Artificial Sequence
  Fc-hIL-2v2
AESKYGPPCPPCPAPEAAGGPSVFLFPPKPKDQLMISRTPEVTCVVVDVSQEDPEVQFNWYVDGVEVHNAKTKPREEQFNSTYRVVSVLTVLHQDWLNGKEYKCKVSNKGLPSSIEKTISKAKGQPREPQVYTLPPSQEEMTKNQVSLTCLVKGFYPSDIAVEWESNGQPENNYKTTPPVLDSDGSFFLYSRLTVDKSRWQEGNVFSCSVLHEALHNHYTQKSLSLSLGGGGGSAPTSSSTKKTQLQLEHLLLDLQMILNGINNYKNPKLTAMLTAKFYMPKKATELKHLQCLEEELKPLEEVLNLAQSKNFHLRPRDLISNINVIVLELKGSETTFMCEYADETATIVEFLNRWITFCQSIISTLT

SEQ ID NO: 12 - protein, 215 aa, Artificial Sequence
  anti-hLAG3(1E09)VH+CH1
QVQLVQSGGDLVKPGGSLRLSCAASGFSFSDHYMNWIRQAPGKGLEWVAYIDTSATYIYYADSVKGRFTISRDNAKNSLYLQMNSLRAEDTAVYYCARDNWGSLDYWGQGALVTVSSASTKGPSVFPLAPCSRSTSESTAALGCLVKDYFPEPVTVSWNSGALTSGVHTFPAVLQSSGLYSLSSVVTVPSSSLGTKTYTCNVDHKPSNTKVDKRV

SEQ ID NO: 13 - protein, 13 aa, Artificial Sequence
  linker 1
AESKYGPPCPPCP

SEQ ID NO: 14 - protein, 216 aa, Artificial Sequence
  hIgG4Fc
APEAAGGPSVFLFPPKPKDQLMISRTPEVTCVVVDVSQEDPEVQFNWYVDGVEVHNAKTKPREEQFNSTYRVVSVLTVLHQDWLNGKEYKCKVSNKGLPSSIEKTISKAKGQPREPQVYTLPPSQEEMTKNQVSLTCLVKGFYPSDIAVEWESNGQPENNYKTTPPVLDSDGSFFLYSRLTVDKSRWQEGNVFSCSVLHEALHNHYTQKSLSLSLG

SEQ ID NO: 15 - protein, 443 aa, Artificial Sequence
  anti-hLAG3(1E09) heavy chain
QVQLVQSGGDLVKPGGSLRLSCAASGFSFSDHYMNWIRQAPGKGLEWVAYIDTSATYIYYADSVKGRFTISRDNAKNSLYLQMNSLRAEDTAVYYCARDNWGSLDYWGQGALVTVSSASTKGPSVFPLAPCSRSTSESTAALGCLVKDYFPEPVTVSWNSGALTSGVHTFPAVLQSSGLYSLSSVVTVPSSSLGTKTYTCNVDHKPSNTKVDKRVESKYGPPCPPCPAPEAAGGPSVFLFPPKPKDQLMISRTPEVTCVVVDVSQEDPEVQFNWYVDGVEVHNAKTKPREEQFNSTYRVVSVLTVLHQDWLNGKEYKCKVSNKGLPSSIEKTISKAKGQPREPQVYTLPPSQEEMTKNQVSLTCLVKGFYPSDIAVEWESNGQPENNYKTTPPVLDSDGSFFLYSRLTVDKSRWQEGNVFSCSVLHEALHNHYTQKSLSLSLG

SEQ ID NO: 16 - protein, 214 aa, Artificial Sequence
  anti-hLAG3(1E09)VL-kappa+ CL
DIQMTQSPSSLSPSVGDRVTITCQASQEISIYLNWYQQKPGKAPKLLIYDASNLETGVPSRFSGSGSGTDFTLTISSLQPEDFATYYCQQTYITPYTFGQGTKLDIKRTVAAPSVFIFPPSDEQLKSGTASVVCLLNNFYPREAKVQWKVDNALQSGNSQESVTEQDSKDSTYSLSSTLTLSKADYEKHKVYACEVTHQGLSSPVTKSFNRGEC

SEQ ID NO: 17 - DNA, 1746 bp, Artificial Sequence
  polynucleotides coding anti-hLAG3HC(1E09, hIgG4Fc)_hIL2v2
caggttcagttggttcagtctggcggcgacctggttaagcctggcggatctctgagactgtcttgtgccgcctccggcttctccttctccgaccactacatgaactggatcagacaggcccctggcaaaggcctggaatgggtcgcctacatcgatacctccgccacctacatctactacgccgactccgtgaagggcagattcaccatctccagagacaacgccaagaactccctgtacctccagatgaacagcctgagagccgaggacaccgccgtgtactactgcgccagagataactggggctccctggattattggggccagggcgctctggtcacagtgtcctctgcttctaccaagggacccagcgtgttccctctggctccttgctccagatccacctccgagtctacagctgctctgggctgcctggtcaaggactactttcctgagcctgtgaccgtgtcctggaactctggcgctctgacatctggcgtgcacacctttccagctgtgctccagtcctccggcctgtactctctgtcctctgtcgtgaccgtgccttcctctagcctgggcaccaagacctacacctgtaatgtggaccacaagccttccaacaccaaggtggacaagcgcgtggccgagtctaagtatggccctccttgtcctccatgtcctgctccagaagctgctggcgggccctccgtgtttctgttccctccaaagcctaaggaccagctgatgatctctcggacacccgaagtgacctgcgtggtggtggatgtgtctcaagaggaccctgaggtgcagttcaattggtacgtggacggcgtggaagtgcacaacgccaagaccaagcctagagaggaacagttcaactccacctacagagtggtgtccgtgctgaccgtgctgcaccaggattggctgaacggcaaagagtacaagtgcaaggtgtccaacaagggcctgccttccagcatcgaaaagaccatctccaaggccaagggccagcctagggaaccccaggtttacaccctgcctccaagccaagaggaaatgaccaagaaccaggtgtccctgacctgcctggtcaagggcttctacccttccgacattgccgtggaatgggagagcaatggccagcctgagaacaactacaagaccacacctcctgtgctggactccgacggctccttctttctgtactcccgcctgaccgtggacaagtccagatggcaagagggcaacgtgttctcctgctctgtgctgcacgaggccctgcacaatcactacacccagaagtccctcagcctgtcccttggcggaggcggtggatccgctcctacctcctccagcaccaagaaaacccagttgcagctggaacatctgctgctggacctccagatgatcctgaacggcatcaacaactacaagaaccccaagctgaccgccatgctgaccgctaagttctacatgcccaagaaggccaccgagcttaagcacctccagtgcctggaagaggaacttaagcccctggaagaagtgctgaatctggcccagtccaagaacttccacctgaggcctcgggacctgatctccaacatcaacgtgatcgtgctggaactcaagggctccgagacaaccttcatgtgcgagtacgccgacgagacagctaccatcgtggaatttctgaatcggtggatcaccttctgccagtccatcatcagcaccctgacc

SEQ ID NO: 18 - DNA, 642 bp, Artificial Sequence
  polynucleotides coding anti-hLAG3(1E09) light chain
gacattcagatgacccagtctccatcctctctgagcccatccgtgggcgacagagtgaccattacctgccaggccagccaagagatctccatctacctgaactggtatcagcagaagcccggcaaggcccctaagctgctgatctacgacgcctccaatctggaaacaggcgtgccctccagattctccggctctggctctggcacagactttaccctgaccatctccagcctccagcctgaggatttcgccacctactactgccagcagacctacatcaccccttacacctttggccagggcaccaagctggacatcaagagaaccgtggccgctccttccgtgttcatcttcccaccttccgacgagcagcttaagtctggcacagcctctgtcgtgtgcctgctgaacaacttctaccctcgggaagccaaggtgcagtggaaggtggacaatgccctccagtccggcaactcccaagagtctgtgaccgagcaggactccaaggacagcacctacagcctgtcctccacactgaccctgtccaaggccgactacgagaagcacaaggtgtacgcctgcgaagtgacccaccagggactgtctagccctgtgaccaagtctttcaaccggggcgagtgc

SEQ ID NO: 19 - protein, 5 aa, Artificial Sequence
  linker 2
GGGGS

SEQ ID NO: 20 - protein, 133 aa, Artificial Sequence
  hIL2v2
APTSSSTKKTQLQLEHLLLDLQMILNGINNYKNPKLTAMLTAKFYMPKKATELKHLQCLEEELKPLEEVLNLAQSKNFHLRPRDLISNINVIVLELKGSETTFMCEYADETATIVEFLNRWITFCQSIISTLT

SEQ ID NO: 21 - protein, 133 aa, Artificial Sequence
  hIL2v3
APTSSSTKKTQLQLEHLLLDLQMILNGINNYKNPKLTAMLTAKFYMPKKATELKHLQCLERELKPLEEVLNLAQSKNFHLRPRDLISNINVIVLELKGSETTFMCEYADETATIVEFLNRWITFCQSIISTLT

SEQ ID NO: 22 - protein, 133 aa, Artificial Sequence [sequence omitted]

SEQ ID NO: 23 - DNA, 1746 bp, Artificial Sequence
  polynucleotides coding anti-hLAG3HC(1E09, hIgG4Fc)_hIL2v3
caggttcagttggttcagtctggcggcgacctggttaagcctggcggatctctgagactgtcttgtgccgcctccggcttctccttctccgaccactacatgaactggatcagacaggcccctggcaaaggcctggaatgggtcgcctacatcgatacctccgccacctacatctactacgccgactccgtgaagggcagattcaccatctccagagacaacgccaagaactccctgtacctccagatgaacagcctgagagccgaggacaccgccgtgtactactgcgccagagataactggggctccctggattattggggccagggcgctctggtcacagtgtcctctgcttctaccaagggacccagcgtgttccctctggctccttgctccagatccacctccgagtctacagctgctctgggctgcctggtcaaggactactttcctgagcctgtgaccgtgtcctggaactctggcgctctgacatctggcgtgcacacctttccagctgtgctccagtcctccggcctgtactctctgtcctctgtcgtgaccgtgccttcctctagcctgggcaccaagacctacacctgtaatgtggaccacaagccttccaacaccaaggtggacaagcgcgtggccgagtctaagtatggccctccttgtcctccatgtcctgctccagaagctgctggcgggccctccgtgtttctgttccctccaaagcctaaggaccagctgatgatctctcggacacccgaagtgacctgcgtggtggtggatgtgtctcaagaggaccctgaggtgcagttcaattggtacgtggacggcgtggaagtgcacaacgccaagaccaagcctagagaggaacagttcaactccacctacagagtggtgtccgtgctgaccgtgctgcaccaggattggctgaacggcaaagagtacaagtgcaaggtgtccaacaagggcctgccttccagcatcgaaaagaccatctccaaggccaagggccagcctagggaaccccaggtttacaccctgcctccaagccaagaggaaatgaccaagaaccaggtgtccctgacctgcctggtcaagggcttctacccttccgacattgccgtggaatgggagagcaatggccagcctgagaacaactacaagaccacacctcctgtgctggactccgacggctccttctttctgtactcccgcctgaccgtggacaagtccagatggcaagagggcaacgtgttctcctgctctgtgctgcacgaggccctgcacaatcactacacccagaagtccctcagcctgtcccttggcggaggcggtggatccgctcctacctcctccagcaccaagaaaacccagttgcagctggaacatctgctgctggacctccagatgatcctgaacggcatcaacaactacaagaaccccaagctgaccgccatgctgaccgctaagttctacatgcccaagaaggccaccgagcttaagcacctccagtgcctggaacgtgaacttaagcccctggaagaagtgctgaatctggcccagtccaagaacttccacctgaggcctcgggacctgatctccaacatcaacgtgatcgtgctggaactcaagggctccgagacaaccttcatgtgcgagtacgccgacgagacagctaccatcgtggaatttctgaatcggtggatcaccttctgccagtccatcatcagcaccctgacc

SEQ ID NO: 24 - protein, 367 aa, Artificial Sequence
  Fc-hIL-2v3
AESKYGPPCPPCPAPEAAGGPSVFLFPPKPKDQLMISRTPEVTCVVVDVSQEDPEVQFNWYVDGVEVHNAKTKPREEQFNSTYRVVSVLTVLHQDWLNGKEYKCKVSNKGLPSSIEKTISKAKGQPREPQVYTLPPSQEEMTKNQVSLTCLVKGFYPSDIAVEWESNGQPENNYKTTPPVLDSDGSFFLYSRLTVDKSRWQEGNVFSCSVLHEALHNHYTQKSLSLSLGGGGGSAPTSSSTKKTQLQLEHLLLDLQMILNGINNYKNPKLTAMLTAKFYMPKKATELKHLQCLERELKPLEEVLNLAQSKNFHLRPRDLISNINVIVLELKGSETTFMCEYADETATIVEFLNRWITFCQSIISTLT

SEQ ID NO: 25 - DNA, 1101 bp, Artificial Sequence
  polynucleotides coding GI-101C2(hIgG4Fc-hIL2v2)
gccgagtctaagtatggccctccttgtcctccatgtcctgctccagaagctgctggcggcccttccgtgtttctgttccctccaaagcctaaggaccagctgatgatctctcggacccctgaagtgacctgcgtggtggtggatgtgtcccaagaggaccctgaggtgcagttcaattggtacgtggacggcgtggaagtgcacaacgccaagaccaagcctagagaggaacagttcaactccacctacagagtggtgtccgtgctgaccgtgctgcaccaggattggctgaacggcaaagagtacaagtgcaaggtgtccaacaagggcctgccttccagcatcgaaaagaccatctccaaggccaagggccagcctagggaaccccaggtttacaccctgcctccaagccaagaggaaatgaccaagaaccaggtgtccctgacctgcctggtcaagggcttctacccttccgacattgccgtggaatgggagagcaatggccagcctgagaacaactacaagaccacacctcctgtgctggactccgacggctccttctttctgtactcccgcctgaccgtggacaagtccagatggcaagagggcaacgtgttctcctgctctgtgctgcacgaggccctgcacaatcactacacccagaagtccctgtctctgtcccttggcggaggcggaggatccgcccctaccagctcctctaccaagaaaacccagctccagttggagcatctgctgctggacctccagatgattctgaacgggatcaacaactataagaaccccaagctgaccgccatgctgaccgctaagttctacatgcccaagaaggccaccgagctgaagcacctccagtgcctggaagaagaactgaagcccctggaagaggtgctgaatctggcccagtccaagaacttccacctgaggccacgggacctgatcagcaacatcaacgtgatcgtgctggaactgaagggctccgagacaacctttatgtgcgagtacgccgacgagacagccaccatcgtggaatttctgaaccggtggatcaccttctgccagagcatcatctccacactgacc

SEQ ID NO: 26 - DNA, 1101 bp, Artificial Sequence
  polynucleotides coding GI-101C3(hIgG4Fc-hIL2v3)
gccgagtctaagtatggccctccttgtcctccatgtcctgctccagaagctgctggcggcccttccgtgtttctgttccctccaaagcctaaggaccagctgatgatctctcggacccctgaagtgacctgcgtggtggtggatgtgtcccaagaggaccctgaggtgcagttcaattggtacgtggacggcgtggaagtgcacaacgccaagaccaagcctagagaggaacagttcaactccacctacagagtggtgtccgtgctgaccgtgctgcaccaggattggctgaacggcaaagagtacaagtgcaaggtgtccaacaagggcctgccttccagcatcgaaaagaccatctccaaggccaagggccagcctagggaaccccaggtttacaccctgcctccaagccaagaggaaatgaccaagaaccaggtgtccctgacctgcctggtcaagggcttctacccttccgacattgccgtggaatgggagagcaatggccagcctgagaacaactacaagaccacacctcctgtgctggactccgacggctccttctttctgtactcccgcctgaccgtggacaagtccagatggcaagagggcaacgtgttctcctgctctgtgctgcacgaggccctgcacaatcactacacccagaagtccctgtctctgtcccttggcggaggcggaggatccgctcctacctccagctccaccaagaaaacccagttgcagctggaacatctgctgctggacctccagatgatcctgaatggcatcaacaattacaagaaccccaagctgaccgccatgctgaccgctaagttctacatgcccaagaaggccaccgagctgaagcacctccagtgcctggaacgggaactgaagcctctggaagaggtgctgaatctggcccagtccaagaacttccacctgaggcctcgggacctgatctccaacatcaacgtgatcgtgctggaactcaagggctccgagacaaccttcatgtgcgagtacgccgacgagacagctaccatcgtggaatttctgaatcggtggatcaccttctgccagtccatcatcagcaccctgacc

SEQ ID NO: 27 - protein, 582 aa, Artificial Sequence
  Anti-hLAG3HC(1E09, hIgG4Fc)_hIL2v2
QVQLVQSGGDLVKPGGSLRLSCAASGFSFSDHYMNWIRQAPGKGLEWVAYIDTSATYIYYADSVKGRFTISRDNAKNSLYLQMNSLRAEDTAVYYCARDNWGSLDYWGQGALVTVSSASTKGPSVFPLAPCSRSTSESTAALGCLVKDYFPEPVTVSWNSGALTSGVHTFPAVLQSSGLYSLSSVVTVPSSSLGTKTYTCNVDHKPSNTKVDKRVAESKYGPPCPPCPAPEAAGGPSVFLFPPKPKDQLMISRTPEVTCVVVDVSQEDPEVQFNWYVDGVEVHNAKTKPREEQFNSTYRVVSVLTVLHQDWLNGKEYKCKVSNKGLPSSIEKTISKAKGQPREPQVYTLPPSQEEMTKNQVSLTCLVKGFYPSDIAVEWESNGQPENNYKTTPPVLDSDGSFFLYSRLTVDKSRWQEGNVFSCSVLHEALHNHYTQKSLSLSLGGGGGSAPTSSSTKKTQLQLEHLLLDLQMILNGINNYKNPKLTAMLTAKFYMPKKATELKHLQCLEEELKPLEEVLNLAQSKNFHLRPRDLISNINVIVLELKGSETTFMCEYADETATIVEFLNRWITFCQSIISTLT

SEQ ID NO: 28 - protein, 582 aa, Artificial Sequence
  Anti-hLAG3HC(1E09, hIgG4Fc)_hIL2v3
QVQLVQSGGDLVKPGGSLRLSCAASGFSFSDHYMNWIRQAPGKGLEWVAYIDTSATYIYYADSVKGRFTISRDNAKNSLYLQMNSLRAEDTAVYYCARDNWGSLDYWGQGALVTVSSASTKGPSVFPLAPCSRSTSESTAALGCLVKDYFPEPVTVSWNSGALTSGVHTFPAVLQSSGLYSLSSVVTVPSSSLGTKTYTCNVDHKPSNTKVDKRVAESKYGPPCPPCPAPEAAGGPSVFLFPPKPKDQLMISRTPEVTCVVVDVSQEDPEVQFNWYVDGVEVHNAKTKPREEQFNSTYRVVSVLTVLHQDWLNGKEYKCKVSNKGLPSSIEKTISKAKGQPREPQVYTLPPSQEEMTKNQVSLTCLVKGFYPSDIAVEWESNGQPENNYKTTPPVLDSDGSFFLYSRLTVDKSRWQEGNVFSCSVLHEALHNHYTQKSLSLSLGGGGGSAPTSSSTKKTQLQLEHLLLDLQMILNGINNYKNPKLTAMLTAKFYMPKKATELKHLQCLERELKPLEEVLNLAQSKNFHLRPRDLISNINVIVLELKGSETTFMCEYADETATIVEFLNRWITFCQSIISTLT

SEQ ID NO: 29 - DNA, 1329 bp, Artificial Sequence
  polynucleotides coding anti-hLAG-3VH(anti-hLAG-3(1E09)VH+CH1) and Fc domain(F02(hIgG4Fc))
caggttcagttggttcagtctggcggcgacctggttaagcctggcggatctctgagactgtcttgtgccgcctccggcttctccttctccgaccactacatgaactggatcagacaggcccctggcaaaggcctggaatgggtcgcctacatcgatacctccgccacctacatctactacgccgactccgtgaagggcagattcaccatctccagagacaacgccaagaactccctgtacctccagatgaacagcctgagagccgaggacaccgccgtgtactactgcgccagagataactggggctccctggattattggggccagggcgctctggtcacagtgtcctctgcttctaccaagggacccagcgtgttccctctggctccttgctccagatccacctccgagtctacagctgctctgggctgcctggtcaaggactactttcctgagcctgtgaccgtgtcctggaactctggcgctctgacatctggcgtgcacacctttccagctgtgctccagtcctccggcctgtactctctgtcctctgtcgtgaccgtgccttcctctagcctgggcaccaagacctacacctgtaatgtggaccacaagccttccaacaccaaggtggacaagcgcgtggagtctaagtatggccctccttgtcctccatgtcctgctccagaagctgctggcgggccctccgtgtttctgttccctccaaagcctaaggaccagctgatgatctctcggacacccgaagtgacctgcgtggtggtggatgtgtctcaagaggaccctgaggtgcagttcaattggtacgtggacggcgtggaagtgcacaacgccaagaccaagcctagagaggaacagttcaactccacctacagagtggtgtccgtgctgaccgtgctgcaccaggattggctgaacggcaaagagtacaagtgcaaggtgtccaacaagggcctgccttccagcatcgaaaagaccatctccaaggccaagggccagcctagggaaccccaggtttacaccctgcctccaagccaagaggaaatgaccaagaaccaggtgtccctgacctgcctggtcaagggcttctacccttccgacattgccgtggaatgggagagcaatggccagcctgagaacaactacaagaccacacctcctgtgctggactccgacggctccttctttctgtactcccgcctgaccgtggacaagtccagatggcaagagggcaacgtgttctcctgctctgtgctgcacgaggccctgcacaatcactacacccagaagtccctcagcctgtcccttggc